European Patent Application EP 4 112 640 A1, published January 4, 2023. Title: Novel single domain antigen binding molecules and their uses. Applicant: NMI Naturwissenschaftliches und Medizinisches Institut an der Universität Tübingen. The sequence listing filed with the application follows.

SEQUENCE LISTING (108 sequences)

SEQ ID NO: 1 - protein, 8 aa, Artificial Sequence
  Nanobody Nb1 CDR1
SGFTFSKL

SEQ ID NO: 2 - protein, 12 aa, Artificial Sequence
  Nanobody Nb1 CDR2
IDSSGDTTDYLA

SEQ ID NO: 3 - protein, 6 aa, Artificial Sequence
  Nanobody Nb1 CDR3
REDPPG

SEQ ID NO: 4 - protein, 8 aa, Artificial Sequence
  Nanobody Nb2 CDR 1
SGFDVDYY

SEQ ID NO: 5 - protein, 12 aa, Artificial Sequence
  Nanobody Nb2 CDR2
IASSDGSTYYAD

SEQ ID NO: 6 - protein, 20 aa, Artificial Sequence
  Nanobody Nb2 CDR3
DATCPYYCSGSVCYLETGMD

SEQ ID NO: 7 - protein, 8 aa, Artificial Sequence
  Nanobody Nb3 CDR1
SGFALEYY

SEQ ID NO: 8 - protein, 12 aa, Artificial Sequence
  Nanobody Nb3 CDR2
MSASGGVINYSE

SEQ ID NO: 9 - protein, 17 aa, Artificial Sequence
  Nanobdy Nb3 CDR3
EKAYYGSSWAECYLMMD

SEQ ID NO: 10 - protein, 116 aa, Artificial Sequence
  Nanobody Nb1
EVQLVESGGGLVQPGGSLRLSCAASGFTFSKLAMSWHREPPGKGREWLADIDSSGDTTDYLASVKGRFTISRDNAKNTLYLQMDSLKSEDTGVYYCASREDPPGYWGQGTQVTVSS

SEQ ID NO: 11 - protein, 130 aa, Artificial Sequence
  Nanobody Nb2
EVQLVESGGGSVQPGGSLRLSCGASGFDVDYYAIGWFRQAPGKEREGVSCIASSDGSTYYADSVKGRFTISRDNAKNTVYLQMNSLKPEDTAVYYCAADATCPYYCSGSVCYLETGMDYWGEGTLVTVSS

SEQ ID NO: 12 - protein, 127 aa, Artificial Sequence
  Nanobody Nb3
HVQLVESGGGLVQPGGSLRLSCAVSGFALEYYAIGWFRQAPGKERERVACMSASGGVINYSESVKGRFTISRDNAKNTVYLQMNTLKPEDTAVYYCAAEKAYYGSSWAECYLMMDYWGKGTLVTVSS

SEQ ID NO: 13 - protein, 15 aa, Artificial Sequence
  HCMVA pp65 aa 109-123
MSIYVYALPLKMLNI

SEQ ID NO: 14 - protein, 17 aa, Artificial Sequence
  HCMV pp65 aa 366-382
HPTFTSQYRIQGKLEYR

SEQ ID NO: 15 - protein, 15 aa, Artificial Sequence
  EBVB9 EBNA2 aa 276-290
PRSPTVFYNIPPMPL

SEQ ID NO: 16 - protein, 14 aa, Artificial Sequence
  EBVB9 EBNA1 aa 514-527
KTSLYNLRRGTALA

SEQ ID NO: 17 - protein, 20 aa, Artificial Sequence
  EBV BXLF2 aa 126-140
LEKQLFYYIGTMLPNTRPHS

SEQ ID NO: 18 - protein, 15 aa, Artificial Sequence
  EBV BRLF1 aa 119-133
DRFFIQAPSNRVMIP

SEQ ID NO: 19 - protein, 15 aa, Artificial Sequence
  EBVB9 EBNA3 aa 381-395
PIFIRRLHRLLLMRA

SEQ ID NO: 20 - protein, 15 aa, Artificial Sequence
  EBVB9 GP350 aa 167-181
STNITAVVRAQGLDV

SEQ ID NO: 21 - protein, 13 aa, Artificial Sequence
  IABAN HEMA aa 306-318
PKYVKQNTLKLAT

SEQ ID NO: 22 - protein, 15 aa, Artificial Sequence
  CMVpp65 aa 510-524
YQEFFWDANDIYRIF

SEQ ID NO: 23 - DNA, 23 bp, Artificial Sequence
  Oligo
gtcctggctgctcttctacaagg

SEQ ID NO: 24 - DNA, 23 bp, Artificial Sequence
  Oligo
ggtacgtgctgttgaactgttcc

SEQ ID NO: 25 - DNA, 33 bp, Artificial Sequence
  Oligo
  misc_feature (7)..(7): n is a, c, g, or t
  misc_feature (10)..(10): n is a, c, g, or t
  misc_feature (25)..(25): n is a, c, g, or t
  misc_feature (28)..(28): n is a, c, g, or t
  misc_feature (31)..(31): n is a, c, g, or t
catggcnsangtgcagctggtggantcnggngg

SEQ ID NO: 26 - DNA, 33 bp, Artificial Sequence
  Oligo
  misc_feature (7)..(7): n is a, c, g, or t
  misc_feature (10)..(10): n is a, c, g, or t
  misc_feature (25)..(25): n is a, c, g, or t
  misc_feature (28)..(28): n is a, c, g, or t
  misc_feature (31)..(31): n is a, c, g, or t
catggcnsangtgcagctgcaggantcnggngg

SEQ ID NO: 27 - DNA, 33 bp, Artificial Sequence
  Oligo
  misc_feature (7)..(7): n is a, c, g, or t
  misc_feature (10)..(10): n is a, c, g, or t
  misc_feature (25)..(25): n is a, c, g, or t
  misc_feature (31)..(31): n is a, c, g, or t
catggcnsangtgcagctggtgganagyggngg

SEQ ID NO: 28 - DNA, 33 bp, Artificial Sequence
  Oligo
  misc_feature (7)..(7): n is a, c, g, or t
  misc_feature (10)..(10): n is a, c, g, or t
  misc_feature (25)..(25): n is a, c, g, or t
  misc_feature (31)..(31): n is a, c, g, or t
catggcnsangtgcagctgcagganagyggngg

SEQ ID NO: 29 - DNA, 38 bp, Artificial Sequence
  Oligo
  misc_feature (22)..(22): n is a, c, g, or t
  misc_feature (25)..(25): n is a, c, g, or t
gtaggcccagccggccatggcnsangtgcagctggtgg

SEQ ID NO: 30 - DNA, 39 bp, Artificial Sequence
  Oligo
  misc_feature (22)..(22): n is a, c, g, or t
  misc_feature (25)..(25): n is a, c, g, or t
gtaggcccagccggccatggcnsangtgcagctgcagga

SEQ ID NO: 31 - DNA, 35 bp, Artificial Sequence
  Oligo
  misc_feature (12)..(12): n is a, c, g, or t
  misc_feature (15)..(15): n is a, c, g, or t
  misc_feature (18)..(18): n is a, c, g, or t
  misc_feature (28)..(28): n is a, c, g, or t
  misc_feature (30)..(30): n is a, c, g, or t
  misc_feature (33)..(33): n is a, c, g, or t
gatgcggccgcnganganacggtgaccngnryncc

SEQ ID NO: 32 - DNA, 35 bp, Artificial Sequence
  Oligo
  misc_feature (12)..(12): n is a, c, g, or t
  misc_feature (15)..(15): n is a, c, g, or t
  misc_feature (18)..(18): n is a, c, g, or t
  misc_feature (28)..(28): n is a, c, g, or t
  misc_feature (30)..(30): n is a, c, g, or t
  misc_feature (33)..(33): n is a, c, g, or t
gatgcggccgcnganganacggtgaccngngancc

SEQ ID NO: 33 - DNA, 35 bp, Artificial Sequence
  Oligo
  misc_feature (12)..(12): n is a, c, g, or t
  misc_feature (15)..(15): n is a, c, g, or t
  misc_feature (18)..(18): n is a, c, g, or t
  misc_feature (28)..(28): n is a, c, g, or t
  misc_feature (33)..(33): n is a, c, g, or t
gatgcggccgcnganganacggtgaccngrctncc

SEQ ID NO: 34 - DNA, 35 bp, Artificial Sequence
  oligo
  misc_feature (15)..(15): n is a, c, g, or t
  misc_feature (18)..(18): n is a, c, g, or t
  misc_feature (28)..(28): n is a, c, g, or t
  misc_feature (30)..(30): n is a, c, g, or t
  misc_feature (33)..(33): n is a, c, g, or t
gatgcggccgcrctnganacggtgaccngnryncc

SEQ ID NO: 35 - DNA, 35 bp, Artificial Sequence
  Oligo
  misc_feature (15)..(15): n is a, c, g, or t
  misc_feature (18)..(18): n is a, c, g, or t
  misc_feature (28)..(28): n is a, c, g, or t
  misc_feature (30)..(30): n is a, c, g, or t
  misc_feature (33)..(33): n is a, c, g, or t
gatgcggccgcrctnganacggtgaccngngancc

SEQ ID NO: 36 - DNA, 35 bp, Artificial Sequence
  Oligo
  misc_feature (15)..(15): n is a, c, g, or t
  misc_feature (18)..(18): n is a, c, g, or t
  misc_feature (28)..(28): n is a, c, g, or t
  misc_feature (33)..(33): n is a, c, g, or t
gatgcggccgcrctnganacggtgaccngrctncc

SEQ ID NO: 37 - DNA, 54 bp, Artificial Sequence
  Primer
acactctttccctacacgacgctcttccgatctggattgttattactcgcggcc

SEQ ID NO: 38 - DNA, 53 bp, Artificial Sequence
  Primer
gactggagttcagacgtgtgctcttccgatctgatcagcttctgttctgcggc

SEQ ID NO: 39 - DNA, 31 bp, Artificial Sequence
  Primer
ggaggatccacaatgaaccggggagtccctt

SEQ ID NO: 40 - DNA, 34 bp, Artificial Sequence
  Primer
ggtctcgagtcaaatggggctacatgtcttctga

SEQ ID NO: 41 - DNA, 34 bp, Artificial Sequence
  Primer
atacccggggccaccatggccaagcctttgtctc

SEQ ID NO: 42 - DNA, 32 bp, Artificial Sequence
  Primer
tatgcgcgcttagccctcccacacataaccag

SEQ ID NO: 43 - DNA, 51 bp, Artificial Sequence
  Primer
gcagtctctcactggagcagcgcgttcggattgactgccaactctgacacc

SEQ ID NO: 44 - DNA, 40 bp, Artificial Sequence
  Primer
gcgcacgcgatcaggcattccctgagtggctgctgggagg

SEQ ID NO: 45 - DNA, 46 bp, Artificial Sequence
  Primer
gcagtctctcactggagcagcgctttccagaaggcctccagcatag

SEQ ID NO: 46 - DNA, 40 bp, Artificial Sequence; identical to SEQ ID NO: 44
  Primer

SEQ ID NO: 47 - DNA, 18 bp, Artificial Sequence
  Primer
cccacatggtccaccccg

SEQ ID NO: 48 - DNA, 25 bp, Artificial Sequence
  Primer
agctagcaccacgatgtctattttg

SEQ ID NO: 49 - DNA, 41 bp, Artificial Sequence
  Oligo
atacgtctcaactctaagaaagtggtgctgggcaaaaaagg

SEQ ID NO: 50 - DNA, 53 bp, Artificial Sequence
  Oligo
tatgaattcagtggtgatggtggtggtggggcagaaccttgatgttggattcc

SEQ ID NO: 51 - protein, 154 aa, Artificial Sequence
  VP1-PepNb
GGGGSGGGGSGGGGSGGGGSGGGGGSAMADVQLQESGGGLVQPGGSLRLSCAASGNIVSIDAAGWFRQAPGKQREPVATILTGGATNYADSVKGRFTISRDNAKNTVYLQMNSLKPEDTAVYYCYAPMIYYGGRYSDYWGQGTQVTVSSGGGGA

SEQ ID NO: 52 - protein, 157 aa, Artificial Sequence
  VP1-CD4-Nb4
GGGGSGGGGSGGGGSGGGGSGGGGSAMAEVQLQESGGALAQPGGSLRLSCAVSGFTFGTYGMGWLRQAPGKGREFVAAINWIHGGEIYADSVKGRFTISKDNAKNTLYLQMDSLKPEDTAVYYCAARSGTSLYTGVDEYQYWGQGTQVTVSSGGGGA

SEQ ID NO: 53 - protein, 149 aa, Artificial Sequence
  VP1-CD4-Nb1
GGGGSGGGGSGGGGSGGGGSGGGGSAMAEVQLVESGGGLVQPGGSLRLSCAASGFTFSKLAMSWHREPPGKGREWLADIDSSGDTTDYLASVKGRFTISRDNAKNTLYLQMDSLKSEDTGVYYCASREDPPGYWGQGTQVTVSSGGGGA

SEQ ID NO: 54 - protein, 160 aa, Artificial Sequence
  VP1-CD4-Nb3
GGGGSGGGGSGGGGSGGGGSGGGGSAMAHVQLVESGGGLVQPGGSLRLSCAVSGFALEYYAIGWFRQAPGKERERVACMSASGGVINYSESVKGRFTISRDNAKNTVYLQMNTLKPEDTAVYYCAAEKAYYGSSWAECYLMMDYWGKGTLVTVSSGGGGA

SEQ ID NO: 55 - protein, 155 aa, Artificial Sequence
  VP1-CD4-Nb1a
GGGGSGGGGSGGGGSGGGGSGGGGGSGGGGSAMAEVQLVESGGGLVQPGGSLRLSCVASGFTFSSSGMTWVRQAPGKGLEWVSDINSGGDTTDYLASVKGRFTISRDNAKNTLYLQMDSLKSEDTGVYYCASREDPPGYWGQGIQVTVSSGGGGA

SEQ ID NO: 56 - protein, 293 aa, Artificial Sequence
  VP1-biCD4-Nb1
GGGGSGGGGSGGGGSGGGGSGGGGSAMAEVQLVESGGGLVQPGGSLRLSCAASGFTFSKLAMSWHREPPGKGREWLADIDSSGDTTDYLASVKGRFTISRDNAKNTLYLQMDSLKSEDTGVYYCASREDPPGYWGQGTQVTVSASGGGGSGGGGSGGGGSGGGGSGGGGSMAEVQLVESGGGLVQPGGSLRLSCAASGFTFSKLAMSWHREPPGKGREWLADIDSSGDTTDYLASVKGRFTISRDNAKNTLYLQMDSLKSEDTGVYYCASREDPPGYWGQGTQVTVSSGGGGA

SEQ ID NO: 57 - protein, 302 aa, Artificial Sequence
  VP1-biPepNB
GGGGSGGGGSGGGGSGGGGSGGGGSAMADVQLQESGGGLVQPGGSLRLSCAASGNIVSIDAAGWFRQAPGKQREPVATILTGGATNYADSVKGRFTISRDNAKNTVYLQMNSLKPEDTAVYYCYAPMIYYGGRYSDYWGQGTQVTVSSASGGGGSGGGGSGGGGSGGGGSGGGGSMADVQLQESGGGLVQPGGSLRLSCAASGNIVSIDAAGWFRQAPGKQREPVATILTGGATNYADSVKGRFTISRDNAKNTVYLQMNSLKPEDTAVYYCYAPMIYYGGRYSDYWGQGTQVTVSSGGGGA

SEQ ID NO: 58 - protein, 598 aa, Artificial Sequence
  AAV2 VP2 Protein (blind and optimized)
MAPGKKRPVEHSPVEPDSSSGTGKAGQQPARKRLNFGQTGDADSVPDPQPLGQPPAAPSGLGTNTMATGSGAPMADNNEGADGVGNSSGNWHCDSTWMGDRVITTSTRTWALPTYNNHLYKQISSQSGASNDNHYFGYSTPWGYFDFNRFHCHFSPRDWQRLINNNWGFRPKRLNFKLFNIQVKEVTQNDGTTTIANNLTSTVQVFTDSEYQLPYVLGSAHQGCLPPFPADVFMVPQYGYLTLNNGSQAVGRSSFYCLEYFPSQMLRTGNNFTFSYTFEDVPFHSSYAHSQSLDRLMNPLIDQFLYYLSRTNTPSGTTTQSRLQFSQAGASDIRDQSRNWLPGPCYRQQRVSKVSADNNNSEFSWTGATKYHLNGRDSLVNPGPAMASHKDDEEKFFPQSGVLIFGKQGSEKTNVDIEKVMITDEEEIRTTNPVATEQYGSVSTNLQAGNAQAATADVNTQGVLPGMVWQDRDVYLQGPIWAKIPHTDGHFHPSPLMGGFGLKHPPPQILIKNTPVPANPSTTFSAAKFASFITQYSTGQVSVEIEWELQKENSKRWNPEIQYTSNYNKSVNVDFTVDTNGVYSEPRPIGTRFLTRNL

SEQ ID NO: 59 - protein, 146 aa, Artificial Sequence
  VP2-PepNb
VPPEPNBMADVQLQESGGGLVQPGGSLRLSCAASGNIVSIDAAGWFRQAPGKQREPVATILTGGATNYADSVKGRFTISRDNAKNTVYLQMNSLKPEDTAVYYCYAPMIYYGGRYSDYWGQGTQVTVSSRGGSGGSGGSGGSGGSR

SEQ ID NO: 60 - protein, 140 aa, Artificial Sequence
  VP2-CD4-Nb4
MAEVQLQESGGALAQPGGSLRLSCAVSGFTFGTYGMGWLRQAPGKGREFVAAINWIHGGEIYADSVKGRFTISKDNAKNTLYLQMDSLKPEDTAVYYCAARSGTSLYTGVDEYQYWGQGTQVTVSSRGGSGGSGGSGGSR

SEQ ID NO: 61 - protein, 140 aa, Artificial Sequence
  VP2-CD4-Nb5
MAEVQLQESGGGLVQAGGSLRLSCKVSGRTFGTYAMGWFRQAPGKEREFVAVISWIKGNTYVADSVLGRFTISRDNARNWLHLQMYSLKPEDTATYYCAASSTVTLPTTLDPYTYWGQGTPVTVSSRGGSGGSGGSGGSR

SEQ ID NO: 62 - protein, 132 aa, Artificial Sequence
  VP2-CD4-Nb1
MAEVQLVESGGGLVQPGGSLRLSCAASGFTFSKLAMSWHREPPGKGREWLADIDSSGDTTDYLASVKGRFTISRDNAKNTLYLQMDSLKSEDTGVYYCASREDPPGYWGQGTQVTVSSRGGSGGSGGSGGSR

SEQ ID NO: 63 - protein, 143 aa, Artificial Sequence
  VP2-CD4-Nb3
MAHVQLVESGGGLVQPGGSLRLSCAVSGFALEYYAIGWFRQAPGKERERVACMSASGGVINYSESVKGRFTISRDNAKNTVYLQMNTLKPEDTAVYYCAAEKAYYGSSWAECYLMMDYWGKGTLVTVSSRGGSGGSGGSGGSR

SEQ ID NO: 64 - protein, 132 aa, Artificial Sequence
  VP2-CD4-Nb1a
MAEVQLVESGGGLVQPGGSLRLSCVASGFTFSSSGMTWVRQAPGKGLEWVSDINSGGDTTDYLASVKGRFTISRDNAKNTLYLQMDSLKSEDTGVYYCASREDPPGYWGQGIQVTVSSRGGSGGSGGSGGSR

SEQ ID NO: 65 - DNA, 27 bp, Artificial Sequence
  Oligo
ccttctagaatggctccgggaaaaaag

SEQ ID NO: 66 - DNA, 27 bp, Artificial Sequence
  oligo
aacggatccttacagattacgagtcag

SEQ ID NO: 67 - DNA, 26 bp, Artificial Sequence
  Oligo
caacgcacaagcagctaccgcagatg

SEQ ID NO: 68 - DNA, 25 bp, Artificial Sequence
  Oligo
cctgcctggaggttggtagatacag

SEQ ID NO: 69 - DNA, 20 bp, Artificial Sequence
  Oligo
agttcctgtattacttgagc

SEQ ID NO: 70 - DNA, 20 bp, Artificial Sequence
  Oligo
ggtcgatgagaggattcatg

SEQ ID NO: 71 - DNA, 26 bp, Artificial Sequence
  Oligo
caacaacagtgaattctcgtggactg

SEQ ID NO: 72 - DNA, 26 bp, Artificial Sequence
  Oligo
ttatccgcagatacctttgatactcg

SEQ ID NO: 73 - DNA, 20 bp, Artificial Sequence
  Oligo
gattcctgactcgtaatctg

SEQ ID NO: 74 - DNA, 20 bp, Artificial Sequence
  Oligo
tggtgccaatggggcgaggc

SEQ ID NO: 75 - DNA, 27 bp, Artificial Sequence
  Oligo
gcgaagcttgccgccatggcagaggtg

SEQ ID NO: 76 - DNA, 27 bp, Artificial Sequence
  Oligo
tgcctcgagaggagacggtgacctggg

SEQ ID NO: 77 - DNA, 27 bp, Artificial Sequence
  Oligo
gcgaagcttgccgccatggcagaggtg

SEQ ID NO: 78 - DNA, 27 bp, Artificial Sequence
  Oligo
ggcctcgagaggaaacggtgaccggag

SEQ ID NO: 79 - DNA, 27 bp, Artificial Sequence
  Oligo
gcgaagcttgccgccatggctgaggtg

SEQ ID NO: 80 - DNA, 27 bp, Artificial Sequence
  Oligo
ggcctcgagatgagacggtgacctggg

SEQ ID NO: 81 - DNA, 27 bp, Artificial Sequence
  Oligo
gcgaagcttgccgccatggcccacgtg

SEQ ID NO: 82 - DNA, 27 bp, Artificial Sequence
  Oligo
ggcctcgagaggagacggtgaccaggg

SEQ ID NO: 83 - DNA, 27 bp, Artificial Sequence
  Oligo
gcgaagcttgccgccatggccgaggtg

SEQ ID NO: 84 - DNA, 26 bp, Artificial Sequence
  Oligo
ggcctcgagaggagacggtgacctgg

SEQ ID NO: 85 - DNA, 30 bp, Artificial Sequence
  Oligo
gcgaagcttgccgccatggctgacgtgcag

SEQ ID NO: 86 - DNA, 28 bp, Artificial Sequence
  Oligo
gcctcgagaggagacggtgacctgggtg

SEQ ID NO: 87 - DNA, 20 bp, Artificial Sequence
  Oligo
tcaggtaaggctgccgatgg

SEQ ID NO: 88 - DNA, 27 bp, Artificial Sequence
  Oligo
tttaaatcatttattgttcaaagatgc

SEQ ID NO: 89 - DNA, 20 bp, Artificial Sequence
  Oligo
tcttccttattggctcgagg

SEQ ID NO: 90 - DNA, 20 bp, Artificial Sequence
  Oligo
taaccatcggcagccatacc

SEQ ID NO: 91 - DNA, 34 bp, Artificial Sequence
  Oligo
acttggagtgtttgttctgctcaagtaatacagg

SEQ ID NO: 92 - DNA, 35 bp, Artificial Sequence
  Oligo
gccgcggcggcggcggcgcgcttcagttttctcag

SEQ ID NO: 93 - DNA, 78 bp, Artificial Sequence
  Oligo
ggcggcggcggcagcggcggcggcggcagcggcggcggcggcagcggcggcggcggcagcggcggcggcggcagcgcg

SEQ ID NO: 94 - DNA, 78 bp, Artificial Sequence
  Oligo
cgcgctgccgccgccgccgctgccgccgccgccgctgccgccgccgccgctgccgccgccgccgctgccgccgccgcc

SEQ ID NO: 95 - DNA, 41 bp, Artificial Sequence
  Oligo
gcggcagcggcggcggcggcagcgctatggctgaggtgcag

SEQ ID NO: 96 - DNA, 41 bp, Artificial Sequence
  Oligo
aactgaagcgcgccgccgccgccgcttgagacggtgacctg

SEQ ID NO: 97 - DNA, 41 bp, Artificial Sequence
  Oligo
gcggcagcggcggcggcggcagcgctatggccgaggtgcag

SEQ ID NO: 98 - DNA, 41 bp, Artificial Sequence
  Oligo
aactgaagcgcgccgccgccgccgctggagacggtgacctg

SEQ ID NO: 99 - DNA, 41 bp, Artificial Sequence
  Oligo
gcggcagcggcggcggcggcagcgctatggcagaggtgcag

SEQ ID NO: 100 - DNA, 41 bp, Artificial Sequence; identical to SEQ ID NO: 98
  Oligo

SEQ ID NO: 101 - DNA, 41 bp, Artificial Sequence
  Oligo
gcggcagcggcggcggcggcagcgctatggcccacgtgcag

SEQ ID NO: 102 - DNA, 41 bp, Artificial Sequence
  Oligo
aactgaagcgcgccgccgccgccgctggagacggtgaccag

SEQ ID NO: 103 - DNA, 41 bp, Artificial Sequence
  Oligo
gcggcagcggcggcggcggcagcgctatggctgacgtgcag

SEQ ID NO: 104 - DNA, 38 bp, Artificial Sequence
  Oligo
aactgaagcgcgccgccgccgccgctggagacggtgac

SEQ ID NO: 105 - DNA, 28 bp, Artificial Sequence
  Oligo
gcggcggcggcggcgcgcttcagttttc

SEQ ID NO: 106 - DNA, 28 bp, Artificial Sequence
  Oligo
aggtacacatctctgtcctgccagacca

SEQ ID NO: 107 - DNA, 20 bp, Artificial Sequence
  Oligo
gcgatctcgatgctttattt

SEQ ID NO: 108 - DNA, 19 bp, Artificial Sequence
  Oligo
agagggagtggactagttt